European Patent Application EP 4 796 637 A1, published August 26, 2026. Title: 一种抗TSLP抗体的药物组合物及其用途. Applicant: 江苏恒瑞医药股份有限公司. The sequence listing filed with the application follows.

SEQUENCE LISTING (12 sequences)

SEQ ID NO: 1 - protein, 5 aa, synthetic construct
  REGION 1..5: note = hu179-33-HCDR1
NYLIE

SEQ ID NO: 2 - protein, 17 aa, synthetic construct
  REGION 1..17: note = hu179-33-HCDR2
VIDPGVGDTNYNENFKG

SEQ ID NO: 3 - protein, 10 aa, synthetic construct
  REGION 1..10: note = hu179-33-HCDR3
EDNTGTAFDY

SEQ ID NO: 4 - protein, 11 aa, synthetic construct
  REGION 1..11: note = hu179-33-LCDR1
KASQSVSSDVT

SEQ ID NO: 5 - protein, 7 aa, synthetic construct
  REGION 1..7: note = hu179-33-LCDR2
YVSEHYT

SEQ ID NO: 6 - protein, 9 aa, synthetic construct
  REGION 1..9: note = hu179-33-LCDR3
QQHHRFPLT

SEQ ID NO: 7 - protein, 119 aa, synthetic construct
  REGION 1..119: note = hu179-33-VH
EVQLVQSGAEVKKPGSSVKVSCKASGYTFSNYLIEWVRQAPGQGLEWIGVIDPGVGDTNYNENFKGRATLTADKSTSTAYIELSSLRSEDTAVYYCAREDNTGTAFDYWGQGTTVTVSS

SEQ ID NO: 8 - protein, 107 aa, synthetic construct
  REGION 1..107: note = hu179-33-VL
SIVMTQTPLSLSVTPGQPASISCKASQSVSSDVTWYLQKPGQSPQLLIYYVSEHYTGVPDRFSGSGYGTDFTLKISRVEAEDVGVYYCQQHHRFPLTFGQGTKLEIK

SEQ ID NO: 9 - protein, 330 aa, synthetic construct
  REGION 1..330: note = hu179-33-CH
ASTKGPSVFPLAPSSKSTSGGTAALGCLVKDYFPEPVTVSWNSGALTSGVHTFPAVLQSSGLYSLSSVVTVPSSSLGTQTYICNVNHKPSNTKVDKKVEPKSCDKTHTCPPCPAPELLGGPSVFLFPPKPKDTLYITREPEVTCVVVDVSHEDPEVKFNWYVDGVEVHNAKTKPREEQYNSTYRVVSVLTVLHQDWLNGKEYKCKVSNKALPAPIEKTISKAKGQPREPQVYTLPPSRDELTKNQVSLTCLVKGFYPSDIAVEWESNGQPENNYKTTPPVLDSDGSFFLYSKLTVDKSRWQQGNVFSCSVMHEALHNHYTQKSLSLSPGK

SEQ ID NO: 10 - protein, 107 aa, synthetic construct [sequence omitted]

SEQ ID NO: 11 - protein, 449 aa, synthetic construct
  CHAIN 1..449: note = hu179-33-HC
EVQLVQSGAEVKKPGSSVKVSCKASGYTFSNYLIEWVRQAPGQGLEWIGVIDPGVGDTNYNENFKGRATLTADKSTSTAYIELSSLRSEDTAVYYCAREDNTGTAFDYWGQGTTVTVSSASTKGPSVFPLAPSSKSTSGGTAALGCLVKDYFPEPVTVSWNSGALTSGVHTFPAVLQSSGLYSLSSVVTVPSSSLGTQTYICNVNHKPSNTKVDKKVEPKSCDKTHTCPPCPAPELLGGPSVFLFPPKPKDTLYITREPEVTCVVVDVSHEDPEVKFNWYVDGVEVHNAKTKPREEQYNSTYRVVSVLTVLHQDWLNGKEYKCKVSNKALPAPIEKTISKAKGQPREPQVYTLPPSRDELTKNQVSLTCLVKGFYPSDIAVEWESNGQPENNYKTTPPVLDSDGSFFLYSKLTVDKSRWQQGNVFSCSVMHEALHNHYTQKSLSLSPGK

SEQ ID NO: 12 - protein, 214 aa, synthetic construct
  CHAIN 1..214: note = hu179-33-LC
SIVMTQTPLSLSVTPGQPASISCKASQSVSSDVTWYLQKPGQSPQLLIYYVSEHYTGVPDRFSGSGYGTDFTLKISRVEAEDVGVYYCQQHHRFPLTFGQGTKLEIKRTVAAPSVFIFPPSDEQLKSGTASVVCLLNNFYPREAKVQWKVDNALQSGNSQESVTEQDSKDSTYSLSSTLTLSKADYEKHKVYACEVTHQGLSSPVTKSFNRGEC